European Patent Application EP 4 632 069 A1, published October 15, 2025. Title: Nucleic acid adjuvant. Applicant: Aomori Yamada Gakuen Educational Corporation. Application JP. The sequence listing filed with the application follows.

SEQUENCE LISTING (8 sequences)

SEQ ID NO: 1 - RNA, 1152 nt, Measles virus
  source 1..1152: mol_type = genomic RNA
accagacaaagctgggaatagaaacttcgtattttcaaagttttctttaatatattgcaaataatgcctaaccacctagggcaggattagggttccggagttcaaccaattagtccttaatcagggcactgtatccgactaacttataccattctttggtctccttgactgttaccttaaaaacccactcacgtttcaaaccccccgtcataataatctgtttctctgacttggatagattcttaacgaagatattctggtgtaagtctagtatcagatagccggacttgagattctggataaacttatttatcaactttctgttcccggagtaaagaagaatgtgcccccaaaatttgcgggtgatcctagatataagttctcgttgcctgctacttaccaatacggggtaagcgtggaacatcccttgttgacttctttggttgtctttgaatcttgccaactccctgtagaggatgagtatagaattaagcaatccatcttgccctgaggcaacatcatggtggatcaattctttgcacagcttaggtccgttaattgccaacccgcaattgatcagcacctgctctataggtgtaagttttttcagagtaggattgatatcacctctactaactgcgtctcccacaattgcttgtatgcagcttagttgcttaatggataggatgtgacctataagtccaggtgaagtcctcacagatgattcaattatctgctgcttaatcttttcaggattcattagccggttagccttgagatctgtcataaccaaataagattcagtagatatgaagttgctgtatctagggtatacaaggttcacttctctataatgagaccctacataacttataaatccctgaacaaaatccccgctgaaaggcataagcttaatcaccagtattgatcctattttgcccaggagcagagccatcgataagatggctgccaattcctctagcttctctatagtatctttgttaggcaagttagtcggatacagtgccctgattaaggactaattggttgaactccggaaccctaatcctgccctaggtggttaggcattatttgcaatatattaaagaaaactttgaaaatacgaagtttctattcccagctttgtctggt

SEQ ID NO: 2 - DNA, 25 bp, synthetic construct
  source 1..25: mol_type = other DNA; note = single-stranded oligodeoxynucleotide
tgctgctgcttgcaagcagcttgat

SEQ ID NO: 3 - RNA, 120 nt, synthetic construct
  source 1..120: mol_type = other RNA
  misc_feature 1..120: note = double-stranded RNA
accagacaaagctgggaatagaaacttcgtattttcaaagttttctttaatatattgcaaataatgcctaaccacctagggcaggattagggttccggagttcaaccaattagtccttaa

SEQ ID NO: 4 - DNA, 145 bp, synthetic construct
  source 1..145: mol_type = other DNA; note = sense strand- chimeric DNA/RNA molecule
  misc_feature 1..25: note = DNA segment
  misc_feature 26..145: note = RNA segment
tgctgctgcttgcaagcagcttgataccagacaaagctgggaatagaaacttcgtattttcaaagttttctttaatatattgcaaataatgcctaaccacctagggcaggattagggttccggagttcaaccaattagtccttaa

SEQ ID NO: 5 - RNA, 120 nt, synthetic construct
  source 1..120: mol_type = other RNA
  misc_feature 1..120: note = antisense strand-synthetic RNA molecule
ttaaggactaattggttgaactccggaaccctaatcctgccctaggtggttaggcattatttgcaatatattaaagaaaactttgaaaatacgaagtttctattcccagctttgtctggt

SEQ ID NO: 6 - RNA, 120 nt, synthetic construct
  source 1..120: mol_type = other RNA; note = double-stranded RNA
aatagaaacttcgtattttcaaagttttctttaatatattgcaaataatgcctaaccacctagggcaggattagggttccggagttcaaccaattagtccttaatcagggcactgtatcc

SEQ ID NO: 7 - DNA, 145 bp, synthetic construct
  source 1..145: mol_type = other DNA; note = sense strand-DNA/RNA chimeric nucleic acid
  misc_feature 1..25: note = DNA segment
  misc_feature 26..145: note = RNA segment
tgctgctgcttgcaagcagcttgataatagaaacttcgtattttcaaagttttctttaatatattgcaaataatgcctaaccacctagggcaggattagggttccggagttcaaccaattagtccttaatcagggcactgtatcc

SEQ ID NO: 8 - RNA, 120 nt, synthetic construct
  source 1..120: mol_type = other RNA; note = antisense strand-synthetic RNA molecule
ggatacagtgccctgattaaggactaattggttgaactccggaaccctaatcctgccctaggtggttaggcattatttgcaatatattaaagaaaactttgaaaatacgaagtttctatt